European Patent Specification EP 3 552 619 B1, published July 30, 2025. Title: FACTOR IX POLYPEPTIDES AND METHODS OF USE THEREOF. Applicant: Bioverativ Therapeutics Inc. Application To be assigned. The sequence listing filed with the application follows.

SEQUENCE LISTING (4 sequences)

SEQ ID NO: 1 - DNA, 7583 bp, Artificial
  FIX-Fc Chain DNA (pSYN-FIX-030)
gcgcgcgttgacattgattattgactagttattaatagtaatcaattacggggtcattagttcatagcccatatatggagttccgcgttacataacttacggtaaatggcccgcctggctgaccgcccaacgacccccgcccattgacgtcaataatgacgtatgttcccatagtaacgccaatagggactttccattgacgtcaatgggtggagtatttacggtaaactgcccacttggcagtacatcaagtgtatcatatgccaagtacgccccctattgacgtcaatgacggtaaatggcccgcctggcattatgcccagtacatgaccttatgggactttcctacttggcagtacatctacgtattagtcatcgctattaccatggtgatgcggttttggcagtacatcaatgggcgtggatagcggtttgactcacggggatttccaagtctccaccccattgacgtcaatgggagtttgttttggcaccaaaatcaacgggactttccaaaatgtcgtaacaactccgccccattgacgcaaatgggcggtaggcgtgtacggtgggaggtctatataagcagagctctctggctaactagagaacccactgcttactggcttatcgaaattaatacgactcactatagggagacccaagcttcgcgacgtacggccgccaccatgcagcgcgtgaacatgatcatggcagaatcaccaggcctcatcaccatctgccttttaggatatctactcagtgctgaatgtacaggtttgtttccttttttaaaatacattgagtatgcttgccttttagatatagaaatatctgatgctgtcttcttcactaaattttgattacatgatttgacagcaatattgaagagtctaacagccagcacgcaggttggtaagtactgtgggaacatcacagattttggctccatgccctaaagagaaattggctttcagattatttggattaaaaacaaagactttcttaagagatgtaaaattttcatgatgttttcttttttgctaaaactaaagaattattcttttacatttcagtttttcttgatcatgaaaacgccaacaaaattctgaatcggccaaagaggtataattcaggtaaattggaagagtttgttcaagggaatctagagagagaatgtatggaagaaaagtgtagttttgaagaagcacgagaagtttttgaaaacactgaaagaacaactgaattttggaagcagtatgttgatggagatcagtgtgagtccaatccatgtttaaatggcggcagttgcaaggatgacattaattcctatgaatgttggtgtccctttggatttgaaggaaagaactgtgaattagatgtaacatgtaacattaagaatggcagatgcgagcagttttgtaaaaatagtgctgataacaaggtggtttgctcctgtactgagggatatcgacttgcagaaaaccagaagtcctgtgaaccagcagtgccatttccatgtggaagagtttctgtttcacaaacttctaagctcacccgtgctgagactgtttttcctgatgtggactatgtaaattctactgaagctgaaaccattttggataacatcactcaaagcacccaatcatttaatgacttcactcgggttgttggtggagaagatgccaaaccaggtcaattcccttggcaggttgttttgaatggtaaagttgatgcattctgtggaggctctatcgttaatgaaaaatggattgtaactgctgcccactgtgttgaaactggtgttaaaattacagttgtcgcaggtgaacataatattgaggagacagaacatacagagcaaaagcgaaatgtgattcgaattattcctcaccacaactacaatgcagctattaataagtacaaccatgacattgcccttctggaactggacgaacccttagtgctaaacagctacgttacacctatttgcattgctgacaaggaatacacgaacatcttcctcaaatttggatctggctatgtaagtggctggggaagagtcttccacaaagggagatcagctttagttcttcagtaccttagagttccacttgttgaccgagccacatgtcttcgatctacaaagttcaccatctataacaacatgttctgtgctggcttccatgaaggaggtagagattcatgtcaaggagatagtgggggaccccatgttactgaagtggaagggaccagtttcttaactggaattattagctggggtgaagagtgtgcaatgaaaggcaaatatggaatatataccaaggtgtcccggtatgtcaactggattaaggaaaaaacaaagctcactgacaaaactcacacatgcccaccgtgcccagctccggaactcctgggcggaccgtcagtcttcctcttccccccaaaacccaaggacaccctcatgatctcccggacccctgaggtcacatgcgtggtggtggacgtgagccacgaagaccctgaggtcaagttcaactggtacgtggacggcgtggaggtgcataatgccaagacaaagccgcgggaggagcagtacaacagcacgtaccgtgtggtcagcgtcctcaccgtcctgcaccaggactggctgaatggcaaggagtacaagtgcaaggtctccaacaaagccctcccagcccccatcgagaaaaccatctccaaagccaaagggcagccccgagaaccacaggtgtacaccctgcccccatcccgggatgagctgaccaagaaccaggtcagcctgacctgcctggtcaaaggcttctatcccagcgacatcgccgtggagtgggagagcaatgggcagccggagaacaactacaagaccacgcctcccgtgttggactccgacggctccttcttcctctacagcaagctcaccgtggacaagagcaggtggcagcaggggaacgtcttctcatgctccgtgatgcatgaggctctgcacaaccactacacgcagaagagcctctccctgtctccgggtaaatgagaattcagacatgataagatacattgatgagtttggacaaaccacaactagaatgcagtgaaaaaaatgctttatttgtgaaatttgtgatgctattgctttatttgtaaccattataagctgcaataaacaagttggggtgggcgaagaactccagcatgagatccccgcgctggaggatcatccagccggcgtcccggaaaacgattccgaagcccaacctttcatagaaggcggcggtggaatcgaaatctcgtagcacgtgtcagtcctgctcctcggccacgaagtgcacgcagttgccggccgggtcgcgcagggcgaactcccgcccccacggctgctcgccgatctcggtcatggccggcccggaggcgtcccggaagttcgtggacacgacctccgaccactcggcgtacagctcgtccaggccgcgcacccacacccaggccagggtgttgtccggcaccacctggtcctggaccgcgctgatgaacagggtcacgtcgtcccggaccacaccggcgaagtcgtcctccacgaagtcccgggagaacccgagccggtcggtccagaactcgaccgctccggcgacgtcgcgcgcggtgagcaccggaacggcactggtcaacttggccatggtttagttcctcaccttgtcgtattatactatgccgatatactatgccgatgattaattgtcaacacgtgctgatcagatccgaaaatggatatacaagctcccgggagctttttgcaaaagcctaggcctccaaaaaagcctcctcactacttctggaatagctcagaggcagaggcggcctcggcctctgcataaataaaaaaaattagtcagccatggggcggagaatgggcggaactgggcggagttaggggcgggatgggcggagttaggggcgggactatggttgctgactaattgagatgcatgctttgcatacttctgcctgctggggagcctggggactttccacacctggttgctgactaattgagatgcatgctttgcatacttctgcctgctggggagcctggggactttccacaccctcgtcgagctagcttcgtgaggctccggtgcccgtcagtgggcagagcgcacatcgcccacagtccccgagaagttggggggaggggtcggcaattgaaccggtgcctagagaaggtggcgcggggtaaactgggaaagtgatgtcgtgtactggctccgcctttttcccgagggtgggggagaaccgtatataagtgcagtagtcgccgtgaacgttctttttcgcaacgggtttgccgccagaacacaggtaagtgccgtgtgtggttcccgcgggcctggcctctttacgggttatggcccttgcgtgccttgaattacttccacctggctccagtacgtgattcttgatcccgagctggagccaggggcgggccttgcgctttaggagccccttcgcctcgtgcttgagttgaggcctggcctgggcgctggggccgccgcgtgcgaatctggtggcaccttcgcgcctgtctcgctgctttcgataagtctctagccatttaaaatttttgatgacctgctgcgacgctttttttctggcaagatagtcttgtaaatgcgggccaggatctgcacactggtatttcggtttttggggccgcgggcggcgacggggcccgtgcgtcccagcgcacatgttcggcgaggcggggcctgcgagcgcggccaccgagaatcggacgggggtagtctcaagctggccggcctgctctggtgcctggcctcgcgccgccgtgtatcgccccgccctgggcggcaaggctggcccggtcggcaccagttgcgtgagcggaaagatggccgcttcccggccctgctccagggggctcaaaatggaggacgcggcgctcgggagagcgggcgggtgagtcacccacacaaaggaaaggggcctttccgtcctcagccgtcgcttcatgtgactccacggagtaccgggcgccgtccaggcacctcgattagttctggagcttttggagtacgtcgtctttaggttggggggaggggttttatgcgatggagtttccccacactgagtgggtggagactgaagttaggccagcttggcacttgatgtaattctccttggaatttgccctttttgagtttggatcttggttcattctcaagcctcagacagtggttcaaagtttttttcttccatttcaggtgtcgtgaacacgtggtcgcggccgcgccgccaccatggagacagacacactcctgctatgggtactgctgctctgggttccaggttccactggtgacaaaactcacacatgcccaccgtgcccagcacctgaactcctgggaggaccgtcagtcttcctcttccccccaaaacccaaggacaccctcatgatctcccggacccctgaggtcacatgcgtggtggtggacgtgagccacgaagaccctgaggtcaagttcaactggtacgtggacggcgtggaggtgcataatgccaagacaaagccgcgggaggagcagtacaacagcacgtaccgtgtggtcagcgtcctcaccgtcctgcaccaggactggctgaatggcaaggagtacaagtgcaaggtctccaacaaagccctcccagcccccatcgagaaaaccatctccaaagccaaagggcagccccgagaaccacaggtgtacaccctgcccccatcccgcgatgagctgaccaagaaccaggtcagcctgacctgcctggtcaaaggcttctatcccagcgacatcgccgtggagtgggagagcaatgggcagccggagaacaactacaagaccacgcctcccgtgttggactccgacggctccttcttcctctacagcaagctcaccgtggacaagagcaggtggcagcaggggaacgtcttctcatgctccgtgatgcatgaggctctgcacaaccactacacgcagaagagcctctccctgtctccgggtaaatgactcgagagatctggccggctgggcccgtttcgaaggtaagcctatccctaaccctctcctcggtctcgattctacgcgtaccggtcatcatcaccatcaccattgagtttaaacccgctgatcagcctcgactgtgccttctagttgccagccatctgttgtttgcccctcccccgtgccttccttgaccctggaaggtgccactcccactgtcctttcctaataaaatgaggaaattgcatcgcattgtctgagtaggtgtcattctattctggggggtggggtggggcaggacagcaagggggaggattgggaagacaatagcaggcatgctggggatgcggtgggctctatggcttctgaggcggaaagaaccagtggcggtaatacggttatccacagaatcaggggataacgcaggaaagaacatgtgagcaaaaggccagcaaaaggccaggaaccgtaaaaaggccgcgttgctggcgtttttccataggctccgcccccctgacgagcatcacaaaaatcgacgctcaagtcagaggtggcgaaacccgacaggactataaagataccaggcgtttccccctagaagctccctcgtgcgctctcctgttccgaccctgccgcttaccggatacctgtccgcctttctcccttcgggaagcgtggcgctttctcatagctcacgctgtaggtatctcagttcggtgtaggtcgttcgctccaagctgggctgtgtgcacgaaccccccgttcagcccgaccgctgcgccttatccggtaactatcgtcttgagtccaacccggtaagacacgacttatcgccactggcagcagccactggtaacaggattagcagagcgaggtatgtaggcggtgctacagagttcttgaagtggtggcctaactacggctacactagaagaacagtatttggtatctgcgctctgctgaagccagttaccttcggaaaaagagttggtagctcttgatccggcaaacaaaccaccgctggtagcggtggtttttttgtttgcaagcagcagattacgcgcagaaaaaaaggatctcaagaagatcctttgatcttttctacggggtctgacgctcagtggaacgaaaactcacgttaagggattttggtcatgacattaacctataaaaataggcgtatcacgaggccctttcgtctcgcgcgtttcggtgatgacggtgaaaacctctgacacatgcagctcccggagacggtcacagcttgtctgtaagcggatgccgggagcagacaagcccgtcagggcgcgtcagcgggtgttggcgggtgtcggggctggcttaactatgcggcatcagagcagattgtactgagagtgcaccatatatgcggtgtgaaataccgcacagatgcgtaaggagaaaataccgcatcaggcgccattcgccattcaggctgcgcaactgttgggaagggcgatcggtgcgggcctcttcgctattacgcca

SEQ ID NO: 2 - protein, 688 aa, Artificial
  FIX-Fc chain
  SIGNAL (-46)..(-19)
  PROPEP (-18)..(-1)
  misc_feature (1)..(642): Mature peptide
  misc_feature (1)..(415): FIX portion
  misc_feature (416)..(642): Fc portion
MQRVNMIMAESPGLITICLLGYLLSAECTVFLDHENANKILNRPKRYNSGKLEEFVQGNLERECMEEKCSFEEAREVFENTERTTEFWKQYVDGDQCESNPCLNGGSCKDDINSYECWCPFGFEGKNCELDVTCNIKNGRCEQFCKNSADNKVVCSCTEGYRLAENQKSCEPAVPFPCGRVSVSQTSKLTRAETVFPDVDYVNSTEAETILDNITQSTQSFNDFTRVVGGEDAKPGQFPWQVVLNGKVDAFCGGSIVNEKWIVTAAHCVETGVKITVVAGEHNIEETEHTEQKRNVIRIIPHHNYNAAINKYNHDIALLELDEPLVLNSYVTPICIADKEYTNIFLKFGSGYVSGWGRVFHKGRSALVLQYLRVPLVDRATCLRSTKFTIYNNMFCAGFHEGGRDSCQGDSGGPHVTEVEGTSFLTGIISWGEECAMKGKYGIYTKVSRYVNWIKEKTKLTDKTHTCPPCPAPELLGGPSVFLFPPKPKDTLMISRTPEVTCVVVDVSHEDPEVKFNWYVDGVEVHNAKTKPREEQYNSTYRVVSVLTVLHQDWLNGKEYKCKVSNKALPAPIEKTISKAKGQPREPQVYTLPPSRDELTKNQVSLTCLVKGFYPSDIAVEWESNGQPENNYKTTPPVLDSDGSFFLYSKLTVDKSRWQQGNVFSCSVMHEALHNHYTQKSLSLSPGK

SEQ ID NO: 3 - DNA, 741 bp, Artificial
  Fc DNA sequence
atggagacagacacactcctgctatgggtactgctgctctgggttccaggttccactggtgacaaaactcacacatgcccaccgtgcccagcacctgaactcctgggaggaccgtcagtcttcctcttccccccaaaacccaaggacaccctcatgatctcccggacccctgaggtcacatgcgtggtggtggacgtgagccacgaagaccctgaggtcaagttcaactggtacgtggacggcgtggaggtgcataatgccaagacaaagccgcgggaggagcagtacaacagcacgtaccgtgtggtcagcgtcctcaccgtcctgcaccaggactggctgaatggcaaggagtacaagtgcaaggtctccaacaaagccctcccagcccccatcgagaaaaccatctccaaagccaaagggcagccccgagaaccacaggtgtacaccctgcccccatcccgcgatgagctgaccaagaaccaggtcagcctgacctgcctggtcaaaggcttctatcccagcgacatcgccgtggagtgggagagcaatgggcagccggagaacaactacaagaccacgcctcccgtgttggactccgacggctccttcttcctctacagcaagctcaccgtggacaagagcaggtggcagcaggggaacgtcttctcatgctccgtgatgcatgaggctctgcacaaccactacacgcagaagagcctctccctgtctccgggtaaa

SEQ ID NO: 4 - protein, 247 aa, Artificial
  Fc chain
  SIGNAL (-20)..(-1)
  misc_feature (1)..(227): Mature Fc sequence
METDTLLLWVLLLWVPGSTGDKTHTCPPCPAPELLGGPSVFLFPPKPKDTLMISRTPEVTCVVVDVSHEDPEVKFNWYVDGVEVHNAKTKPREEQYNSTYRVVSVLTVLHQDWLNGKEYKCKVSNKALPAPIEKTISKAKGQPREPQVYTLPPSRDELTKNQVSLTCLVKGFYPSDIAVEWESNGQPENNYKTTPPVLDSDGSFFLYSKLTVDKSRWQQGNVFSCSVMHEALHNHYTQKSLSLSPGK